European Patent Specification EP 3 374 391 B1, published April 17, 2024. Title: ANTIBODY MOLECULE-DRUG CONJUGATES AND USES THEREOF. Applicant: VISTERRA, INC. The sequence listing filed with the application follows.

SEQUENCE LISTING (167 sequences)

SEQ ID NO: 1 - protein, 118 aa, Artificial Sequence
  source: /note="Description of Artificial Sequence: Synthetic polypeptide"
EVQLQQSGPVLVKPGASVKMSCKASGYTFTDHYINWVKQSHGKSLEWIGGIYPYHGITKYNRNFKDKATLTVDKSSSTAYMELNSLTSELSAVYYCASGGSRRYFDVWGTGTTVTVSS

SEQ ID NO: 2 - protein, 120 aa, Artificial Sequence
  source: /note="Description of Artificial Sequence: Synthetic polypeptide"
EVQLVESGGGLVQPGGSLRLSCAASGFTFSDYYMTWVRQAPGKGLEWVGLIRNKRNGDTAEYSASVKGRFTISRDDSKNSLYLQMNSLKTEDTAVYYCARQGRGYTLDYWGQGTLVTVSS

SEQ ID NO: 3 - protein, 120 aa, Artificial Sequence
  source: /note="Description of Artificial Sequence: Synthetic polypeptide"
EVQLVESGGGLVQPGGSLRLSCAASGFTFSDYWMTWVRQAPGKGLEWVGLIRAKANGDTAEYSASVKGRFTISRDDSKNSLYLQMNSLKTEDTAVYYCARQGRGYTLDYWGQGTLVTVSS

SEQ ID NO: 4 - protein, 116 aa, Artificial Sequence
  source: /note="Description of Artificial Sequence: Synthetic polypeptide"
QVQLQQPGAELVKPGASVKMSCKASGYTFTSYWITWVKQRPGQGLEWIGDIYPGSGSTNYNEKFKSKATLTVDTSSSTAYMQLSSLTSEDSAVYYCARGSYSLDYWGQGTTLTVSS

SEQ ID NO: 5 - protein, 117 aa, Artificial Sequence
  source: /note="Description of Artificial Sequence: Synthetic polypeptide"
EVQLQQSVAELVRPGASVKLSCTASGFNIKNTYMHWVKQRPEQGLEWIGRIDPANGNTKYAPKFQGKATITADTSSNTAYLQLSSLTSEDTAIYYCAPSNYHAMDYWGQGTSVTVSS

SEQ ID NO: 6 - protein, 117 aa, Artificial Sequence
  source: /note="Description of Artificial Sequence: Synthetic polypeptide"
DVQLQESGPGLVKPSQSLSLTCSVTGYSITSGYYWNWIRQFPGNKLEWMGYISYDGSNNYNPSLKNRISITRDTSKNQFFLKLNSVTTEDTATYYCARWNGNYFDYWGQGTTLTVSS

SEQ ID NO: 7 - protein, 120 aa, Artificial Sequence
  source: /note="Description of Artificial Sequence: Synthetic polypeptide"
EVQLQQSGPVLVKPGASVKMSCKASGYTFTDYYMNWVKQSHGKSLEWIGVINPYNGGTSYNQKFKGKATLTVDKSSSTAYMELNSLTSEDSAVYYCARTRQLGLRWFAYWGQGTLVTVSA

SEQ ID NO: 8 - protein, 112 aa, Artificial Sequence
  source: /note="Description of Artificial Sequence: Synthetic polypeptide"
DVVMTQTPLSLPVSLGDQASISCRSSQRLVHSNGNTYLHWYLQKPGQSPKLLIYKVSNRFSGVPDRFSGSGSGTDFTLKISRVEAEDLGVYFCSQSTHVPYTFGGGTKLEIK

SEQ ID NO: 9 - protein, 107 aa, Artificial Sequence
  source: /note="Description of Artificial Sequence: Synthetic polypeptide"
DIQMTQSPSSVSASVGDRVTITCRASQNINIWLSWYQQKPGKAPKLLIYKASNLHTGVPSRFSGSGSGTDFTLTISSLQPEDFATYYCLQGQSYPRTFGGGTKVEIK

SEQ ID NO: 10 - protein, 112 aa, Artificial Sequence
  source: /note="Description of Artificial Sequence: Synthetic polypeptide"
DIVMTQAAPSVPVTPGESVSISCRSSKSLLHSNGNTYLYWFLQRPGQSPQRLIYYMSNLASGVPDRFSGRGSGTDFTLRISRVEAEDVGVYYCMQSLEYPLTFGAGTKLELK

SEQ ID NO: 11 - protein, 112 aa, Artificial Sequence
  source: /note="Description of Artificial Sequence: Synthetic polypeptide"
DIVMTQAAPSVPVTPGESVSISCRSSKSLLHSNGNTYLYWFLQRPGQSPQLLIYRMSNLASGVPDRFSGSGSGTAFTLRISRVEAEDVGVYYCMQHLEYPYTFGGGTKLEIK

SEQ ID NO: 12 - protein, 112 aa, Artificial Sequence
  source: /note="Description of Artificial Sequence: Synthetic polypeptide"
DIVMSQSPSSLAVSAGEKVTMSCKSSQSLLNSRTRKNYLAWYQQKPGQSPKLLIYWASTRESGVPDRFTGSGSGTDFTLTISSVQAEDLAVYYCKQSYNLWTFGGGTKLEIK

SEQ ID NO: 13 - protein, 107 aa, Artificial Sequence
  source: /note="Description of Artificial Sequence: Synthetic polypeptide"
DIQMTQSPASQSASLGESVTITCLASQTIGTWLAWYQQKPGKSPQLLIYAATSLADGVPSRFSGSGSGTKFSFKISSLQAEDFVSYYCQQLYSTPWTFGGGTKLEIK

SEQ ID NO: 14 - protein, 7 aa, Artificial Sequence
  source: /note="Description of Artificial Sequence: Synthetic peptide"
GYTFTDH

SEQ ID NO: 15 - protein, 6 aa, Artificial Sequence
  source: /note="Description of Artificial Sequence: Synthetic peptide"
YPYHGI

SEQ ID NO: 16 - protein, 9 aa, Artificial Sequence
  source: /note="Description of Artificial Sequence: Synthetic peptide"
GGSRRYFDV

SEQ ID NO: 17 - protein, 5 aa, Artificial Sequence
  source: /note="Description of Artificial Sequence: Synthetic peptide"
DHYIN

SEQ ID NO: 18 - protein, 17 aa, Artificial Sequence
  source: /note="Description of Artificial Sequence: Synthetic peptide"
GIYPYHGITKYNRNFKD

SEQ ID NO: 19 - protein, 7 aa, Artificial Sequence
  source: /note="Description of Artificial Sequence: Synthetic peptide"
GFTFSDY

SEQ ID NO: 20 - protein, 8 aa, Artificial Sequence
  source: /note="Description of Artificial Sequence: Synthetic peptide"
RNKRNGDT

SEQ ID NO: 21 - protein, 9 aa, Artificial Sequence
  source: /note="Description of Artificial Sequence: Synthetic peptide"
QGRGYTLDY

SEQ ID NO: 22 - protein, 5 aa, Artificial Sequence
  source: /note="Description of Artificial Sequence: Synthetic peptide"
DYYMT

SEQ ID NO: 23 - protein, 19 aa, Artificial Sequence
  source: /note="Description of Artificial Sequence: Synthetic peptide"
LIRNKRNGDTAEYSASVKG

SEQ ID NO: 24 - protein, 19 aa, Artificial Sequence
  source: /note="Description of Artificial Sequence: Synthetic peptide"
GSGSGSGSGSGSLPETGGG

SEQ ID NO: 25 - protein, 8 aa, Artificial Sequence
  source: /note="Description of Artificial Sequence: Synthetic peptide"
RAKANGDT

SEQ ID NO: 26 - protein, 19 aa, Artificial Sequence
  source: /note="Description of Artificial Sequence: Synthetic peptide"
PGGGGSGGGGSLPETGGSG

SEQ ID NO: 27 - protein, 5 aa, Artificial Sequence
  source: /note="Description of Artificial Sequence: Synthetic peptide"
DYWMT

SEQ ID NO: 28 - protein, 19 aa, Artificial Sequence
  source: /note="Description of Artificial Sequence: Synthetic peptide"
LIRAKANGDTAEYSASVKG

SEQ ID NO: 29 - protein, 7 aa, Artificial Sequence
  source: /note="Description of Artificial Sequence: Synthetic peptide"
GYTFTSY

SEQ ID NO: 30 - protein, 6 aa, Artificial Sequence
  source: /note="Description of Artificial Sequence: Synthetic peptide"
YPGSGS

SEQ ID NO: 31 - protein, 7 aa, Artificial Sequence
  source: /note="Description of Artificial Sequence: Synthetic peptide"
GSYSLDY

SEQ ID NO: 32 - protein, 5 aa, Artificial Sequence
  source: /note="Description of Artificial Sequence: Synthetic peptide"
SYWIT

SEQ ID NO: 33 - protein, 17 aa, Artificial Sequence
  source: /note="Description of Artificial Sequence: Synthetic peptide"
DIYPGSGSTNYNEKFKS

SEQ ID NO: 34 - protein, 7 aa, Artificial Sequence
  source: /note="Description of Artificial Sequence: Synthetic peptide"
GFNIKNT

SEQ ID NO: 35 - protein, 6 aa, Artificial Sequence
  source: /note="Description of Artificial Sequence: Synthetic peptide"
DPANGN

SEQ ID NO: 36 - protein, 8 aa, Artificial Sequence
  source: /note="Description of Artificial Sequence: Synthetic peptide"
SNYHAMDY

SEQ ID NO: 37 - protein, 5 aa, Artificial Sequence
  source: /note="Description of Artificial Sequence: Synthetic peptide"
NTYMH

SEQ ID NO: 38 - protein, 17 aa, Artificial Sequence
  source: /note="Description of Artificial Sequence: Synthetic peptide"
RIDPANGNTKYAPKFQG

SEQ ID NO: 39 - protein, 8 aa, Artificial Sequence
  source: /note="Description of Artificial Sequence: Synthetic peptide"
GYSITSGY

SEQ ID NO: 40 - protein, 5 aa, Artificial Sequence
  source: /note="Description of Artificial Sequence: Synthetic peptide"
SYDGS

SEQ ID NO: 41 - protein, 8 aa, Artificial Sequence
  source: /note="Description of Artificial Sequence: Synthetic peptide"
WNGNYFDY

SEQ ID NO: 42 - protein, 6 aa, Artificial Sequence
  source: /note="Description of Artificial Sequence: Synthetic peptide"
SGYYWN

SEQ ID NO: 43 - protein, 16 aa, Artificial Sequence
  source: /note="Description of Artificial Sequence: Synthetic peptide"
YISYDGSNNYNPSLKN

SEQ ID NO: 44 - protein, 7 aa, Artificial Sequence
  source: /note="Description of Artificial Sequence: Synthetic peptide"
GYTFTDY

SEQ ID NO: 45 - protein, 6 aa, Artificial Sequence
  source: /note="Description of Artificial Sequence: Synthetic peptide"
NPYNGG

SEQ ID NO: 46 - protein, 11 aa, Artificial Sequence
  source: /note="Description of Artificial Sequence: Synthetic peptide"
TRQLGLRWFAY

SEQ ID NO: 47 - protein, 5 aa, Artificial Sequence
  source: /note="Description of Artificial Sequence: Synthetic peptide"
DYYMN

SEQ ID NO: 48 - protein, 17 aa, Artificial Sequence
  source: /note="Description of Artificial Sequence: Synthetic peptide"
VINPYNGGTSYNQKFKG

SEQ ID NO: 49 - protein, 16 aa, Artificial Sequence
  source: /note="Description of Artificial Sequence: Synthetic peptide"
RSSQRLVHSNGNTYLH

SEQ ID NO: 50 - protein, 7 aa, Artificial Sequence
  source: /note="Description of Artificial Sequence: Synthetic peptide"
KVSNRFS

SEQ ID NO: 51 - protein, 9 aa, Artificial Sequence
  source: /note="Description of Artificial Sequence: Synthetic peptide"
SQSTHVPYT

SEQ ID NO: 52 - protein, 11 aa, Artificial Sequence
  source: /note="Description of Artificial Sequence: Synthetic peptide"
RASQNINIWLS

SEQ ID NO: 53 - protein, 7 aa, Artificial Sequence
  source: /note="Description of Artificial Sequence: Synthetic peptide"
KASNLHT

SEQ ID NO: 54 - protein, 9 aa, Artificial Sequence
  source: /note="Description of Artificial Sequence: Synthetic peptide"
LQGQSYPRT

SEQ ID NO: 55 - protein, 16 aa, Artificial Sequence
  source: /note="Description of Artificial Sequence: Synthetic peptide"
RSSKSLLHSNGNTYLY

SEQ ID NO: 56 - protein, 7 aa, Artificial Sequence
  source: /note="Description of Artificial Sequence: Synthetic peptide"
YMSNLAS

SEQ ID NO: 57 - protein, 9 aa, Artificial Sequence
  source: /note="Description of Artificial Sequence: Synthetic peptide"
MQSLEYPLT

SEQ ID NO: 58 - protein, 16 aa, Artificial Sequence
  source: /note="Description of Artificial Sequence: Synthetic peptide"
RSSKSLLHSNGNTYLY

SEQ ID NO: 59 - protein, 7 aa, Artificial Sequence
  source: /note="Description of Artificial Sequence: Synthetic peptide"
RMSNLAS

SEQ ID NO: 60 - protein, 9 aa, Artificial Sequence
  source: /note="Description of Artificial Sequence: Synthetic peptide"
MQHLEYPYT

SEQ ID NO: 61 - protein, 17 aa, Artificial Sequence
  source: /note="Description of Artificial Sequence: Synthetic peptide"
KSSQSLLNSRTRKNYLA

SEQ ID NO: 62 - protein, 7 aa, Artificial Sequence
  source: /note="Description of Artificial Sequence: Synthetic peptide"
WASTRES

SEQ ID NO: 63 - protein, 8 aa, Artificial Sequence
  source: /note="Description of Artificial Sequence: Synthetic peptide"
KQSYNLWT

SEQ ID NO: 64 - protein, 11 aa, Artificial Sequence
  source: /note="Description of Artificial Sequence: Synthetic peptide"
LASQTIGTWLA

SEQ ID NO: 65 - protein, 7 aa, Artificial Sequence
  source: /note="Description of Artificial Sequence: Synthetic peptide"
AATSLAD

SEQ ID NO: 66 - protein, 9 aa, Artificial Sequence
  source: /note="Description of Artificial Sequence: Synthetic peptide"
QQLYSTPWT

SEQ ID NO: 67 - protein, 16 aa, Artificial Sequence
  source: /note="Description of Artificial Sequence: Synthetic peptide"
ALWKTLLKKVLKAAAK

SEQ ID NO: 68 - protein, 29 aa, Artificial Sequence
  source: /note="Description of Artificial Sequence: Synthetic peptide"
RGLRRLGRKIAHGVKKYGPTVLRIIRIAG

SEQ ID NO: 69 - protein, 22 aa, Artificial Sequence
  source: /note="Description of Artificial Sequence: Synthetic peptide"
GIGKFLKKAKKFGKAFVKILKK

SEQ ID NO: 70 - protein, 26 aa, Artificial Sequence
  source: /note="Description of Artificial Sequence: Synthetic peptide"
ALWKTLLKKVLKAAAKGGGGSGGGGS

SEQ ID NO: 71 - protein, 32 aa, Artificial Sequence
  source: /note="Description of Artificial Sequence: Synthetic polypeptide"
GIGKFLKKAKKFGKAFVKILKKGGGGSGGGGS

SEQ ID NO: 72 - protein, 11 aa, Artificial Sequence
  source: /note="Description of Artificial Sequence: Synthetic peptide"
KKLLKWLKKLL

SEQ ID NO: 73 - protein, 22 aa, Artificial Sequence
  source: /note="Description of Artificial Sequence: Synthetic peptide"
GIGKFLKKAKKFGKAFVKILKK

SEQ ID NO: 74 - protein, 37 aa, Artificial Sequence
  source: /note="Description of Artificial Sequence: Synthetic polypeptide"
RLGNFFRKAKKKIGRGLKKIGQKIKDFLGNLVPRTES

SEQ ID NO: 75 - protein, 32 aa, Artificial Sequence
  source: /note="Description of Artificial Sequence: Synthetic polypeptide"
GGGGSGGGGSGIGKFLKKAKKFGKAFVKILKK

SEQ ID NO: 76 - protein, 32 aa, Artificial Sequence
  source: /note="Description of Artificial Sequence: Synthetic polypeptide"
GLRKRLRKFRNKIKEKLKKIGQKIQGLLPKLA

SEQ ID NO: 77 - protein, 26 aa, Artificial Sequence
  source: /note="Description of Artificial Sequence: Synthetic peptide"
GGGGSGGGGSALWKTLLKKVLKAAAK

SEQ ID NO: 78 - protein, 26 aa, Artificial Sequence
  source: /note="Description of Artificial Sequence: Synthetic peptide"
GWKKWFNRAKKVGKTVGGLAVDHYLG

SEQ ID NO: 79 - protein, 30 aa, Artificial Sequence
  source: /note="Description of Artificial Sequence: Synthetic polypeptide"
GAFGNFLKGVAKKAGLKILSIAQCKLFGTC

SEQ ID NO: 80 - protein, 32 aa, Artificial Sequence
  source: /note="Description of Artificial Sequence: Synthetic polypeptide"
GGGRGLRRLGRKIAHGVKKYGPTVLRIIRIAG

SEQ ID NO: 81 - DNA, 354 bp, Artificial Sequence
  source: /note="Description of Artificial Sequence: Synthetic polynucleotide"
gaggtccagctgcagcagtctggacctgtgctggtgaagcctggggcttcagtgaagatgtcctgtaaggcttctggatacacattcactgaccactatataaactgggtgaagcagagccatggaaagagccttgagtggattggaggtatttatccttaccacggtattactaagtacaaccggaatttcaaggacaaggccacattgactgttgacaagtcctccagcacagcctacatggagctcaacagcctgacatctgaactctctgcagtctattactgtgcaagcgggggaagtcgccggtacttcgatgtctggggcacagggaccacggtcaccgtctcctca

SEQ ID NO: 82 - DNA, 360 bp, Artificial Sequence
  source: /note="Description of Artificial Sequence: Synthetic polynucleotide"
gaagtgcagctcgtggaatctggaggaggacttgtgcaacctggaggttccctgcgactgtcgtgtgccgcatccggtttcaccttttccgactactacatgacctgggtcagacaggcgccggggaagggactggagtgggtcggcttgatccgcaacaagaggaacggcgatactgctgaatactcggccagcgtgaaggggcggttcaccatctcgagagatgacagcaagaactccctgtacctccaaatgaactccctgaaaaccgaggacactgcggtgtactactgcgcccgccagggtcgcggctacacgctggactattggggccagggcaccctggtcactgtgtcaagc

SEQ ID NO: 83 - DNA, 360 bp, Artificial Sequence
  source: /note="Description of Artificial Sequence: Synthetic polynucleotide"
gaagtgcagctcgtggaatctggaggaggacttgtgcaacctggaggttccctgcgactgtcgtgtgccgcatccggtttcaccttttccgactactggatgacctgggtcagacaggcgccggggaagggactggagtgggtcggcttgatccgcgccaaggcgaacggcgatactgctgaatactcggccagcgtgaaggggcggttcaccatctcgagagatgacagcaagaactccctgtacctccaaatgaactccctgaaaaccgaggacactgcggtgtactactgcgcccgccagggtcgcggctacacgctggactattggggccagggcaccctggtcactgtgtcaagc

SEQ ID NO: 84 - DNA, 348 bp, Artificial Sequence
  source: /note="Description of Artificial Sequence: Synthetic polynucleotide"
caggtccaactgcagcagcctggggctgagcttgtgaagcctggggcttcagtgaagatgtcctgcaaggcttctggctacaccttcaccagctactggataacctgggtgaagcagaggcctggacaaggccttgagtggattggagatatttatcctggtagtggtagtactaactacaatgagaagttcaagagcaaggccacactgactgtagacacatcctccagcacagcctacatgcagctcagcagcctgacatctgaggactctgcggtctattactgtgcaagaggtagctactcccttgactactggggccaaggcaccactctcacagtctcctca

SEQ ID NO: 85 - DNA, 351 bp, Artificial Sequence
  source: /note="Description of Artificial Sequence: Synthetic polynucleotide"
gaggttcagctgcagcagtctgtggcagagcttgtgaggccaggggcctcagtcaagttgtcctgcacagcttctggcttcaacattaaaaacacctatatgcactgggtgaagcagaggcctgaacagggcctggagtggattggaaggattgatcctgcgaatggtaatactaaatatgccccgaagttccagggcaaggccactataactgcagacacatcctccaacacagcctacctgcagctcagcagcctgacatctgaggacactgccatctattactgtgctcctagtaactaccatgctatggactactggggtcaaggaacctcagtcaccgtctcctca

SEQ ID NO: 86 - DNA, 351 bp, Artificial Sequence
  source: /note="Description of Artificial Sequence: Synthetic polynucleotide"
gatgtacagcttcaggagtcaggacctggcctcgtgaaaccttctcagtctctgtctctcacctgctctgtcactggctactccatcaccagtggttattactggaactggatccggcagtttccaggaaacaaactggaatggatgggctacataagctacgatggtagcaataactacaacccatctctcaaaaatcgaatctccatcactcgtgacacatctaagaaccagtttttcctgaagttgaattctgtgactactgaggacacagccacatattactgtgcaagatggaatggtaactactttgactactggggccaaggcaccactctcacagtctcctca

SEQ ID NO: 87 - DNA, 360 bp, Artificial Sequence
  source: /note="Description of Artificial Sequence: Synthetic polynucleotide"
gaggtccagctgcaacagtctggacctgtgctggtgaagcctggggcttcagtgaagatgtcctgtaaggcttctggatacacattcactgactactatatgaactgggtgaagcagagccatggaaagagccttgagtggattggagttattaatccttacaacggtggtactagctacaaccagaagttcaagggcaaggccacattgactgttgacaagtcctccagcacagcctacatggagctcaacagcctgacatctgaggactctgcagtctattactgtgcaagaaccagacagctcgggctacgttggtttgcttactggggccaagggactctggtcactgtctctgca

SEQ ID NO: 88 - DNA, 336 bp, Artificial Sequence
  source: /note="Description of Artificial Sequence: Synthetic polynucleotide"
gatgttgtgatgacccaaactccactctccctgcctgtcagtcttggagatcaagcctccatctcttgcagatctagtcagagacttgtacacagtaatggaaacacctatttacattggtacctgcagaagccaggccagtctccaaagctcctgatctacaaagtttccaaccgattttctggggtcccagacaggttcagtggcagtggatcagggacagatttcacactcaagatcagcagagtggaggctgaggatctgggagtttatttctgctctcaaagtacacatgttccgtacacgttcggaggggggaccaagctggaaataaaa

SEQ ID NO: 89 - DNA, 321 bp, Artificial Sequence
  source: /note="Description of Artificial Sequence: Synthetic polynucleotide"
gacatccagatgactcagtccccgtcctcagtctccgcatccgtgggagatcgcgtgacgattacttgccgggcgtcgcagaacatcaacatctggctgtcgtggtaccagcagaagcccgggaaggctccgaagctgctgatctacaaggcctcaaacttgcacaccggcgtgccttcccgcttttctggttcgggctccgggactgacttcaccctgaccatcagcagcctgcaacccgaggacttcgccacctattactgcctccaaggacagtcctacccaagaaccttcggcggaggaaccaaggtcgaaatcaaa

SEQ ID NO: 90 - DNA, 336 bp, Artificial Sequence
  source: /note="Description of Artificial Sequence: Synthetic polynucleotide"
gatattgtgatgactcaggctgcaccctctgtacctgtcactcctggagagtcagtatccatctcctgcaggtctagtaagagtcttctgcatagtaatggcaacacttacttgtattggttcctgcagaggccaggccagtctcctcagcgcctgatatattatatgtccaaccttgcctcaggagtcccagacaggttcagtggcagagggtcaggaactgatttcacactgagaatcagtagagtggaggctgaggatgtgggtgtttattactgtatgcaaagtctagaatatcctctcacgttcggtgctgggaccaagctggagctgaaa

SEQ ID NO: 91 - DNA, 336 bp, Artificial Sequence
  source: /note="Description of Artificial Sequence: Synthetic polynucleotide"
gatattgtgatgactcaggctgcaccctctgtacctgtcactcctggagagtcagtatccatctcctgcaggtctagtaagagtctcctgcatagtaatggcaacacttacttgtattggttcctgcagaggccaggccagtctcctcagctcctgatatatcggatgtccaaccttgcctcaggagtcccagacaggttcagtggcagtgggtcaggaactgctttcacactgagaatcagtagagtggaggctgaggatgtgggtgtttattactgtatgcaacatctagaatatccgtacacgttcggaggggggaccaagctggaaataaaa

SEQ ID NO: 92 - DNA, 336 bp, Artificial Sequence
  source: /note="Description of Artificial Sequence: Synthetic polynucleotide"
gacattgtgatgtcacagtctccatcctccctggctgtgtcagcaggagagaaggtcactatgagctgcaaatccagtcagagtctgctcaacagtagaacccgaaagaactacttggcttggtaccagcagaaaccagggcagtctcctaaactgctgatctactgggcatccactagggaatctggggtccctgatcgcttcacaggcagtggatctgggacagatttcactctcaccatcagcagtgtgcaggctgaagacctggcagtttattactgcaagcaatcttataatctgtggacgttcggtggaggcaccaagctggaaatcaaa

SEQ ID NO: 93 - DNA, 321 bp, Artificial Sequence
  source: /note="Description of Artificial Sequence: Synthetic polynucleotide"
gacattcagatgacccagtctcctgcctcccagtctgcatctctgggagaaagtgtcaccatcacatgcctggcaagtcagaccattggtacatggttagcatggtatcagcagaaaccagggaaatctcctcagctcctgatttatgctgcaaccagcttggcagatggggtcccatcaaggttcagtggtagtggatctggcacaaaattttctttcaagatcagcagcctacaggctgaagattttgtaagttattactgtcaacaactttacagtactccgtggacgttcggtggaggcaccaagctggaaatcaaa

SEQ ID NO: 94 - protein, 23 aa, Artificial Sequence
  source: /note="Description of Artificial Sequence: Synthetic peptide"
GIGKHVGKALKGLKGLLKGLGES

SEQ ID NO: 95 - protein, 26 aa, Artificial Sequence
  source: /note="Description of Artificial Sequence: Synthetic peptide"
GRRKRKWLRRIGKGVKIIGGAALDHL

SEQ ID NO: 96 - protein, 27 aa, Artificial Sequence
  source: /note="Description of Artificial Sequence: Synthetic peptide"
GGLRSLGRKILRAWKKYGPQATPATRQ

SEQ ID NO: 97 - protein, 14 aa, Artificial Sequence
  source: /note="Description of Artificial Sequence: Synthetic peptide"
IKWKKLLRAAKRIL

SEQ ID NO: 98 - protein, 19 aa, Artificial Sequence
  source: /note="Description of Artificial Sequence: Synthetic peptide"
IGKKWKRIVKRIKKFLRKL

SEQ ID NO: 99 - protein, 12 aa, Artificial Sequence
  source: /note="Description of Artificial Sequence: Synthetic peptide"
ILGKIWKIKKLF

SEQ ID NO: 100 - protein, 37 aa, Artificial Sequence
  source: /note="Description of Artificial Sequence: Synthetic polypeptide"
RLGDILQKAREKIEGGLKKLVQKIKDFFGKFAPRTES

SEQ ID NO: 101 - protein, 30 aa, Artificial Sequence
  source: /note="Description of Artificial Sequence: Synthetic polypeptide"
GGGGRFKRFRKKFKKLFKKLSPVIPLLHLG

SEQ ID NO: 102 - protein, 27 aa, Artificial Sequence
  source: /note="Description of Artificial Sequence: Synthetic peptide"
GRFKRFRKKFKKLFKKLSPVIPLLHLG

SEQ ID NO: 103 - protein, 119 aa, Artificial Sequence
  source: /note="Description of Artificial Sequence: Synthetic polypeptide"
EVKLVESGGDLVKPGGSLRLSCAASEFTFSDYAMSWVRQTPAKRLEWVAYISSDGDSTYYPDNIKGRFTISRDNAKNTLYLQMNSLRSEDTAMYFCAREIRLRGYFDVWGAGTTVTVSS

SEQ ID NO: 104 - protein, 111 aa, Artificial Sequence
  source: /note="Description of Artificial Sequence: Synthetic polypeptide"
DIVLTQSPASLAVSLGQRATISCRASESVFGHGISPMHWYQQKPGQPPKLLIYRASNLKFGIPARFSGSGSRTDFTLTINPVEADDVATYYCQQSNEYPRTFGGGTKLEIK

SEQ ID NO: 105 - protein, 7 aa, Artificial Sequence
  source: /note="Description of Artificial Sequence: Synthetic peptide"
EFTFSDY

SEQ ID NO: 106 - protein, 6 aa, Artificial Sequence
  source: /note="Description of Artificial Sequence: Synthetic peptide"
SSDGDS

SEQ ID NO: 107 - protein, 10 aa, Artificial Sequence
  source: /note="Description of Artificial Sequence: Synthetic peptide"
EIRLRGYFDV

SEQ ID NO: 108 - protein, 5 aa, Artificial Sequence
  source: /note="Description of Artificial Sequence: Synthetic peptide"
DYAMS

SEQ ID NO: 109 - protein, 17 aa, Artificial Sequence
  source: /note="Description of Artificial Sequence: Synthetic peptide"
YISSDGDSTYYPDNIKG

SEQ ID NO: 110 - protein, 15 aa, Artificial Sequence
  source: /note="Description of Artificial Sequence: Synthetic peptide"
RASESVFGHGISPMH

SEQ ID NO: 111 - protein, 7 aa, Artificial Sequence
  source: /note="Description of Artificial Sequence: Synthetic peptide"
RASNLKF

SEQ ID NO: 112 - protein, 9 aa, Artificial Sequence
  source: /note="Description of Artificial Sequence: Synthetic peptide"
QQSNEYPRT

SEQ ID NO: 113 - DNA, 357 bp, Artificial Sequence
  source: /note="Description of Artificial Sequence: Synthetic polynucleotide"
gaagtgaagttggtggagtctgggggagacttggtgaaacctggagggtccctgagactctcctgtgcagcctctgaattcactttcagtgattatgccatgtcttgggttcgccagactccggcgaagaggctggagtgggtcgcatacattagtagtgatggtgatagtacctactatccggacaatattaagggccgattcaccatctccagagacaatgccaagaacaccctatacctgcaaatgaacagtctgaggtctgaggacacggccatgtatttttgtgcaagagaaatacggctaagggggtacttcgatgtctggggcgcagggaccacggtcaccgtctcctca

SEQ ID NO: 114 - DNA, 333 bp, Artificial Sequence
  source: /note="Description of Artificial Sequence: Synthetic polynucleotide"
gacattgtgctgacccaatctccagcttctttggctgtgtctctagggcagagggccaccatatcctgcagagccagtgaaagtgtttttggtcatggcattagtcctatgcactggtaccagcagaaaccaggacagccacccaaactcctcatctatcgtgcatccaacctaaaatttgggatccctgccaggttcagtggcagtgggtctaggacagacttcaccctcaccattaatcctgtggaggctgatgatgttgcaacctattactgtcagcaaagtaatgaatatcctcggacgttcggtggaggcaccaagctggagatcaaa

SEQ ID NO: 115 - protein, 119 aa, Artificial Sequence
  source: /note="Description of Artificial Sequence: Synthetic polypeptide"
EVKLVESGGGLVQPGGSLRLSCSASEFTFSDYAMSWVRQAPGKGLEWVSYISSDGDSTYYPDNIKGRFTISRDNSKNTLYVQMSSLRAEDTAVYFCAREIRLRGYFDVWGQGTTVTVSS

SEQ ID NO: 116 - protein, 119 aa, Artificial Sequence
  source: /note="Description of Artificial Sequence: Synthetic polypeptide"
EVKLVESGGGLVKPGGSLRLSCAASEFTFSDYAMSWVRQAPGKRLEWVAYISSDGDSIYYPDNIKGRFTISRDNAKNSLYLQMNSLRAEDTAMYFCAREIRLRGYFDVWGQGTTVTVSS

SEQ ID NO: 117 - protein, 119 aa, Artificial Sequence
  source: /note="Description of Artificial Sequence: Synthetic polypeptide"
EVKLVESGGGLVQPGGSLRLSCAASEFTFSDYAMSWVRQAPGKRLEWVAYISSDGDSTYYPDSVKGRFTISRDNAKNSLYLQMNSLRAEDTAMYFCAREIRLRGYFDVWGQGTTVTVSS

SEQ ID NO: 118 - protein, 119 aa, Artificial Sequence
  source: /note="Description of Artificial Sequence: Synthetic polypeptide"
EVKLVESGEGLVQPGGSLRLSCAASEFTFSDYAMSWVRQAPGKRLEWVAYISSDGDSTYYPDNIKGRFTISRDNSKNTLYLQMGSLRAEDMAMYFCAREIRLRGYFDVWGQGTTVTVSS

SEQ ID NO: 119 - protein, 111 aa, Artificial Sequence
  source: /note="Description of Artificial Sequence: Synthetic polypeptide"
EIVMTQSPATLSVSPGERATLSCRASESVFGHGISPLHWYQQKPGQAPKLLIYRASNRKTGIPARFSGSGSGTEFTLTISSLQSEDFAVYYCQQSNEYPRTFGGGTKVEIK

SEQ ID NO: 120 - protein, 111 aa, Artificial Sequence
  source: /note="Description of Artificial Sequence: Synthetic polypeptide"
DIQMTQSPSTLSASVGDRVTITCRASESVFGHGISPLHWYQQKPGKAPKLLIYRASNLKFGVPSRFSGSGSGTEFTLTISSLQPDDFATYYCQQSNEYPRTFGGGTKVEIK

SEQ ID NO: 121 - protein, 111 aa, Artificial Sequence
  source: /note="Description of Artificial Sequence: Synthetic polypeptide"
EIVMTQSPATLSVSPGERATLSCRASESVFGHGISPLHWYQQKPGQPPRLLIYRASNRKTGIPARFSGSGSGTEFTLTISSLQSEDFAVYYCQQSNEYPRTFGGGTKVEIK

SEQ ID NO: 122 - protein, 111 aa, Artificial Sequence
  source: /note="Description of Artificial Sequence: Synthetic polypeptide"
DIQMTQSPSTLSASVGDRVTITCRASESVFGHGISPLHWYQQKPGKAPKLLIYRASNLKFGVPSRFSGSGSRTDFTLTISSLQPDDFATYYCQQSNEYPRTFGGGTKVEIK

SEQ ID NO: 123 - protein, 111 aa, Artificial Sequence
  source: /note="Description of Artificial Sequence: Synthetic polypeptide"
DIQMTQSPSTLSASVGDRVTITCRASESVFGHGISPLHWYQQKPGKAPKLLIYRASNLKFGIPSRFSGSGSRTDFTLTISSLQPDDFATYYCQQSNEYPRTFGGGTKVEIK

SEQ ID NO: 124 - protein, 111 aa, Artificial Sequence
  source: /note="Description of Artificial Sequence: Synthetic polypeptide"
DIQMTQSPSTLSASVGDRVTITCRASESVFGHGISPLHWYQQKPGQPPKLLIYRASNLKFGIPSRFSGSGSGTEFTLTISSLQPDDFATYYCQQSNEYPRTFGGGTKVEIK

SEQ ID NO: 125 - protein, 111 aa, Artificial Sequence
  source: /note="Description of Artificial Sequence: Synthetic polypeptide"
DIVLTQSPSTLSASVGDRVTITCRASESVFGHGISPMHWYQQKPGKAPKLLIYRASNLKFGVPSRFSGSGSGTEFTLTISSLQPDDFATYYCQQSNEYPRTFGGGTKVEIK

SEQ ID NO: 126 - protein, 111 aa, Artificial Sequence
  source: /note="Description of Artificial Sequence: Synthetic polypeptide"
DIQMTQSPSTLSASVGDRVTITCRASESVFGHGISPLHWYQQKPGKAPKLLIYRASNLKFGIPARFSGSGSGTEFTLTISSLQPDDFATYYCQQSNEYPRTFGGGTKVEIK

SEQ ID NO: 127 - protein, 111 aa, Artificial Sequence
  source: /note="Description of Artificial Sequence: Synthetic polypeptide"
DIVLTQSPASLAVSLGQRATISCRASESIFGHGISPMHWYQQKPGQPPKLLIYRASNLKFGIPARFSGSGSRTDFTLTINPVEADDVATYYCQQSNEYPRTFGGGTKLEIK

SEQ ID NO: 128 - protein, 111 aa, Artificial Sequence
  source: /note="Description of Artificial Sequence: Synthetic polypeptide"
DIVLTQSPASLAVSLGQRATISCRASESVFGHGISPMHWYQQKPGQPPKLLIYRASSLKFGIPARFSGSGSRTDFTLTINPVEADDVATYYCQQSNEYPRTFGGGTKLEIK

SEQ ID NO: 129 - protein, 111 aa, Artificial Sequence
  source: /note="Description of Artificial Sequence: Synthetic polypeptide"
DIVLTQSPASLAVSLGQRATISCRASESVFGHGISPMHWYQQKPGQPPKLLIYRASNLKSGIPARFSGSGSRTDFTLTINPVEADDVATYYCQQSNEYPRTFGGGTKLEIK

SEQ ID NO: 130 - protein, 111 aa, Artificial Sequence
  source: /note="Description of Artificial Sequence: Synthetic polypeptide"
DIVMTQSPATLSVSPGERATLSCRASESVFGHGISPLHWYQQKPGQAPKLLIYRASNLKTGIPARFSGSGSRTDFTLTISSLQSEDFATYYCQQSNEYPRTFGGGTKVEIK

SEQ ID NO: 131 - protein, 111 aa, Artificial Sequence
  source: /note="Description of Artificial Sequence: Synthetic polypeptide"
EIVMTQSPATLSVSPGERATISCRASESVFGHGISPLHWYQQKPGQAPKLLIYRASNRKTGIPARFSGSGSGTEFTLTISPVQSEDFAVYYCQQSNEYPRTFGGGTKLEIK

SEQ ID NO: 132 - protein, 111 aa, Artificial Sequence
  source: /note="Description of Artificial Sequence: Synthetic polypeptide"
DIQMTQSPSTLSASVGDRVTITCRASESIFGHGISPLHWYQQKPGKAPKLLIYRASNLKSGIPSRFSGSGSRTEFTLTISSLQPDDFATYYCQQSNEYPRTFGGGTKVEIK

SEQ ID NO: 133 - protein, 111 aa, Artificial Sequence
  source: /note="Description of Artificial Sequence: Synthetic polypeptide"
DIQMTQSPSTLSASVGDRVTITCRASESIFGHGISPLHWYQQKPGKAPKLLIYRASNLKSGVPSRFSGSGSRTEFTLTISSLQPDDFATYYCQQSNEYPRTFGGGTKVEIK

SEQ ID NO: 134 - protein, 111 aa, Artificial Sequence
  source: /note="Description of Artificial Sequence: Synthetic polypeptide"
DIQMTQSPSTLSASVGDRVTITCRASESIFGHGISPLHWYQQKPGKAPKLLIYRASNLKSGVPARFSGSGSRTEFTLTISSLQPDDFATYYCQQSNEYPRTFGGGTKVEIK

SEQ ID NO: 135 - protein, 111 aa, Artificial Sequence
  source: /note="Description of Artificial Sequence: Synthetic polypeptide"
DIQMTQSPSTLSASVGDRVTITCRASESVFGHGISPLHWYQQKPGKAPKLLIYRASNLKSGVPSRFSGSGSRTEFTLTISSLQPDDFATYYCQQSNEYPRTFGGGTKVEIK

SEQ ID NO: 136 - protein, 111 aa, Artificial Sequence
  source: /note="Description of Artificial Sequence: Synthetic polypeptide"
DIQMTQSPSTLSASVGDRVTITCRASESIFGHGISPLHWYQQKPGKAPKLLIYRASNLKSGVPSRFSGSGSRTDFTLTISSLQPDDFATYYCQQSNEYPRTFGGGTKVEIK

SEQ ID NO: 137 - protein, 111 aa, Artificial Sequence
  source: /note="Description of Artificial Sequence: Synthetic polypeptide"
DIQMTQSPSTLSASVGDRVTITCRASESIFGHGISPLHWYQQKPGKAPKLLIYRASNLKSGIPSRFSGSGSRTDFTLTISSLQPDDFATYYCQQSNEYPRTFGGGTKVEIK

SEQ ID NO: 138 - protein, 15 aa, Artificial Sequence
  source: /note="Description of Artificial Sequence: Synthetic peptide"
RASESVFGHGISPLH

SEQ ID NO: 139 - protein, 7 aa, Artificial Sequence
  source: /note="Description of Artificial Sequence: Synthetic peptide"
RASNRKT

SEQ ID NO: 140 - protein, 15 aa, Artificial Sequence
  source: /note="Description of Artificial Sequence: Synthetic peptide"
RASESIFGHGISPMH

SEQ ID NO: 141 - protein, 7 aa, Artificial Sequence
  source: /note="Description of Artificial Sequence: Synthetic peptide"
RASSLKF

SEQ ID NO: 142 - protein, 7 aa, Artificial Sequence
  source: /note="Description of Artificial Sequence: Synthetic peptide"
RASNLKS

SEQ ID NO: 143 - protein, 7 aa, Artificial Sequence
  source: /note="Description of Artificial Sequence: Synthetic peptide"
RASNLKT

SEQ ID NO: 144 - protein, 15 aa, Artificial Sequence
  source: /note="Description of Artificial Sequence: Synthetic peptide"
RASESIFGHGISPLH

SEQ ID NO: 145 - protein, 17 aa, Artificial Sequence
  source: /note="Description of Artificial Sequence: Synthetic peptide"
YISSDGDSIYYPDNIKG

SEQ ID NO: 146 - protein, 17 aa, Artificial Sequence
  source: /note="Description of Artificial Sequence: Synthetic peptide"
YISSDGDSTYYPDSVKG

SEQ ID NO: 147 - protein, 40 aa, Artificial Sequence
  source: /note="Description of Artificial Sequence: Synthetic polypeptide"
GGGLLGDFFRKSKEKIGKEFKRIVQRIKDFLRNLVPRTES

SEQ ID NO: 148 - protein, 29 aa, Artificial Sequence
  source: /note="Description of Artificial Sequence: Synthetic peptide"
GGGKWKSFIKKLTKAAKKVVTTAKKPLIV

SEQ ID NO: 149 - protein, 18 aa, Artificial Sequence
  source: /note="Description of Artificial Sequence: Synthetic peptide"
GGGVNWKKILGKIIKVVK

SEQ ID NO: 150 - protein, 32 aa, Artificial Sequence
  source: /note="Description of Artificial Sequence: Synthetic polypeptide"
GGGTLISWIKNKRKQRPRVSRRRRRRGGRRRR

SEQ ID NO: 151 - protein, 29 aa, Artificial Sequence
  source: /note="Description of Artificial Sequence: Synthetic peptide"
GGGGIGAILKVLATGLPTLISWIKNKRKQ

SEQ ID NO: 152 - protein, 35 aa, Artificial Sequence
  source: /note="Description of Artificial Sequence: Synthetic polypeptide"
GGGGLRKRLRKFRNKIKEKLKKIGQKIQGLLPKLA

SEQ ID NO: 153 - protein, 31 aa, Artificial Sequence
  source: /note="Description of Artificial Sequence: Synthetic polypeptide"
GGGGLRRLGRKIAHGIKKYGPTILRIIRIAG

SEQ ID NO: 154 - protein, 32 aa, Artificial Sequence
  source: /note="Description of Artificial Sequence: Synthetic polypeptide"
GGGRGLRRLGRKIAHGVKKYGPTVLRIIKKYG

SEQ ID NO: 155 - protein, 37 aa, Artificial Sequence
  source: /note="Description of Artificial Sequence: Synthetic polypeptide"
GGGKRFKKFFKKLKNSVKKRAKKFFKKPRVIGVSIPF

SEQ ID NO: 156 - protein, 33 aa, Artificial Sequence
  source: /note="Description of Artificial Sequence: Synthetic polypeptide"
GGGKFFRKLKKSVKKRAKEFFKKPRVIGVSIPF

SEQ ID NO: 157 - protein, 30 aa, Artificial Sequence
  source: /note="Description of Artificial Sequence: Synthetic polypeptide"
GSGSGSGSGSGSGSGSGSGSGSGSGSGSGS

SEQ ID NO: 158 - protein, 22 aa, Artificial Sequence
  source: /note="Description of Artificial Sequence: Synthetic peptide"
GIGKFLKKAKKCGKACVKILKK

SEQ ID NO: 159 - protein, 30 aa, Artificial Sequence
  source: /note="Description of Artificial Sequence: Synthetic polypeptide"
GGGGRCKRFRKKCKKLFKKLSPVIPLLHLG

SEQ ID NO: 160 - protein, 5 aa, Staphylococcus aureus
  MOD_RES (3)..(3): Any amino acid
LPXTG

SEQ ID NO: 161 - protein, 5 aa, Staphylococcus pyogenes
  MOD_RES (3)..(3): Any amino acid
LPXTA

SEQ ID NO: 162 - protein, 5 aa, Staphylococcus sp.
LPETG

SEQ ID NO: 163 - protein, 25 aa, Artificial Sequence
  source: /note="Description of Artificial Sequence: Synthetic peptide"
GGGGIGKFLKKAKKFGKAFVKILKK

SEQ ID NO: 164 - protein, 11 aa, Artificial Sequence
  source: /note="Description of Artificial Sequence: Synthetic peptide"
  MOD_RES (4)..(4): D-Dab
  MOD_RES (5)..(6): Dab
  MISC_FEATURE (5)..(11): Cyclic
  MOD_RES (7)..(7): D-Leu
  MOD_RES (9)..(10): Dab
GGGXXXLFXXL

SEQ ID NO: 165 - protein, 17 aa, Artificial Sequence
  source: /note="Description of Artificial Sequence: Synthetic peptide"
  VARIANT (9)..(9): /replace="Thr"
  VARIANT (14)..(14): /replace="Ser"
  VARIANT (15)..(15): /replace="Val"
  MISC_FEATURE (1)..(17): /note="Variant residues given in the sequence have no preference with respect to those in the annotations for variant positions"
YISSDGDSIYYPDNIKG

SEQ ID NO: 166 - protein, 15 aa, Artificial Sequence
  source: /note="Description of Artificial Sequence: Synthetic peptide"
  VARIANT (6)..(6): /replace="Ile"
  VARIANT (14)..(14): /replace="Leu"
  MISC_FEATURE (1)..(15): /note="Variant residues given in the sequence have no preference with respect to those in the annotations for variant positions"
RASESVFGHGISPMH

SEQ ID NO: 167 - protein, 7 aa, Artificial Sequence
  source: /note="Description of Artificial Sequence: Synthetic peptide"
  VARIANT (4)..(4): /replace="Ser"
  VARIANT (5)..(5): /replace="Arg"
  VARIANT (7)..(7): /replace="Thr" or "Ser"
  MISC_FEATURE (1)..(7): /note="Variant residues given in the sequence have no preference with respect to those in the annotations for variant positions"
RASNLKF